European Patent Application EP 4 137 150 A1, published February 22, 2023. Title: BRACHYURY DELETION MUTANTS, NON-YEAST VECTORS ENCODING BRACHYURY DELETION MUTANTS, AND THEIR USE. Applicant: THE UNITED STATES OF AMERICA, AS REPRESENTED BY THE SECRETARY, DEPARTMENT OF HEALTH AND HUMAN SERVICES. The sequence listing filed with the application follows.

SEQUENCE LISTING (3 sequences)

SEQ ID NO: 1 - protein, 435 aa, Artificial Sequence
  Synthetic
MSSPGTESAGKSLQYRVDHLLSAVENELQAGSEKGDPTERELRVGLEESELWLRFKELTNEMIVTKNGRRMFPVLKVNVSGLDPNAMYSFLLDFVAADNHRWKYVNGEWVPGGKPEPQAPSCVYIHPDSPNFGAHWMKAPVSFSKVKLTNKLNGGGQIMLNSLHKYEPRIHIVRVGGPQRMITSHCFPETQFIAVTAYQNEEITALKIKYNPFAKAFLDAKERSDHKEMMEEPGDSQQPGYSQWGWLLPGTSTLCPPANPHPQFGGALSLPSTHSCDRYPTLRSHRSSPYPSPYAHRNNSPTYSDNSPACLSMLQSHDNWSSLGMPAHPSMLPVSHNASPPTSSSQYPSLWSVSNGAVTPGSQAAAVSNGLGAQFFRGSPAHYTPLTHPVSAPSSSGSPLYEGAAAATDIVDSQYDAAAQGRLIASWTPVSPPSM

SEQ ID NO: 2 - protein, 435 aa, Artificial Sequence
  Synthetic
  MISC_FEATURE (246)..(254): agonist peptide
MSSPGTESAGKSLQYRVDHLLSAVENELQAGSEKGDPTERELRVGLEESELWLRFKELTNEMIVTKNGRRMFPVLKVNVSGLDPNAMYSFLLDFVAADNHRWKYVNGEWVPGGKPEPQAPSCVYIHPDSPNFGAHWMKAPVSFSKVKLTNKLNGGGQIMLNSLHKYEPRIHIVRVGGPQRMITSHCFPETQFIAVTAYQNEEITALKIKYNPFAKAFLDAKERSDHKEMMEEPGDSQQPGYSQWGWLLPGTSTVCPPANPHPQFGGALSLPSTHSCDRYPTLRSHRSSPYPSPYAHRNNSPTYSDNSPACLSMLQSHDNWSSLGMPAHPSMLPVSHNASPPTSSSQYPSLWSVSNGAVTPGSQAAAVSNGLGAQFFRGSPAHYTPLTHPVSAPSSSGSPLYEGAAAATDIVDSQYDAAAQGRLIASWTPVSPPSM

SEQ ID NO: 3 - protein, 410 aa, Artificial Sequence
  Synthetic
  MISC_FEATURE (229)..(229): wherein Xaa is Ser or Val
MSSPGTESAGKSLQYRVDHLLSAVENELQAGSEKGDPTERELRVGLEESELWLRFKELTNEMIVTKNGRRMFPVLKVNVSGLDPNAMYSFLLDFVAADNHRWKYVNGEWVPGGKPEPQAPSCVYIHPDSPNFGAHWMKAPVSFSKVKLTNKLNGGGQIMLNSLHKYEPRIHIVRVGGPQRMITSHCFPETQFIAVTARSDHKEMMEEPGDSQQPGYSQWGWLLPGTSTXCPPANPHPQFGGALSLPSTHSCDRYPTLRSHRSSPYPSPYAHRNNSPTYSDNSPACLSMLQSHDNWSSLGMPAHPSMLPVSHNASPPTSSSQYPSLWSVSNGAVTPGSQAAAVSNGLGAQFFRGSPAHYTPLTHPVSAPSSSGSPLYEGAAAATDIVDSQYDAAAQGRLIASWTPVSPPSM